European Patent Application EP 4 635 980 A1, published October 22, 2025. Title: UNI-TABS specific antibody. Applicant: MEDIGENE IMMUNOTHERAPIES GMBH. Application EP. The sequence listing filed with the application follows.

SEQUENCE LISTING (90 sequences)

SEQ ID NO: 1 - protein, 12 aa, synthetic construct
DKGEVPKDRFSA

SEQ ID NO: 2 - protein, 241 aa, synthetic construct
MDMRVPAQLLGLLLLWLSGARCDVLMTQTPVSLPVSLGGQVSISCRSSQSLVHSDGNTYLHWYLQKPGQSPQLLIYRVSNRFSGVPDRFTGSGSGTDFTLKISRVEPEDLGVYYCLQSTHFPLTFGSGTKLEIKRADAAPTVSIFPPSTEQLATGGASVVCLMNNFYPRDISVKWKIDGTERRDGVLDSVTDQDSKDSTYSMSSTLSLTKADYESHNLYTCEVVHKTSSSPVVKSFNRNEC

SEQ ID NO: 3 - protein, 16 aa, synthetic construct
RSSQSLVHSDGNTYLH

SEQ ID NO: 4 - protein, 7 aa, synthetic construct
RVSNRFS

SEQ ID NO: 5 - protein, 9 aa, synthetic construct
LQSTHFPLT

SEQ ID NO: 6 - protein, 460 aa, synthetic construct
MEFGLSWVFLVALFRGVQCEVQLEESGGGLVQPGRSMKLSCAASGFTFSDYGMAWVLQGPTKGLEWVASISYDGNRPYYRDSVKGRFTISRDNAKSTLYLQMESLRSEDTATYYCVKDLFEIGDFDYWGQGVMVTVSSAETTAPSVYPLAPGTALKSNSMVTLGCLVKGYFPEPVTVTWNSGALSSGVHTFPAVLQSGLYTLTSSVTVPSSTWSSQAVTCNVAHPASSTKVDKKIVPRECNPCGCTGSEVSSVFIFPPKTKDVLTITLTPKVTCVVVDISQNDPEVRFSWFIDDVEVHTAQTHAPEKQSNSTLRSVSELPIVHRDWLNGKTFKCKVNSGAFPAPIEKSISKPEGTPRGPQVYTMAPPKEEMTQSQVSITCMVKGFYPPDIYTEWKMNGQPQENYKNTPPTMDTDGSYFLYSKLNVKKETWQQGNTFTCSVLHEGLHNHHTEKSLSHSPGK

SEQ ID NO: 7 - protein, 7 aa, synthetic construct
GFTFSDY

SEQ ID NO: 8 - protein, 6 aa, synthetic construct
SYDGNR

SEQ ID NO: 9 - protein, 10 aa, synthetic construct
DLFEIGDFDY

SEQ ID NO: 10 - DNA, 726 bp, synthetic construct
  source 1..726: mol_type = other DNA
atggacatgagagtgcctgctcaactgctgggcctgctgctgctttggcttagcggagccagatgcgacgtgctgatgacccagacacctgtgtctctgccagtgtctctcggaggccaggtgtccatcagctgtagaagcagccagagcctggtgcacagcgacggcaatacctacctgcactggtatctgcagaagcccggccagtctcctcagctgctgatctacagagtgtccaaccggttcagcggcgtgcccgatagattcacaggatctggcagcggcaccgacttcaccctgaagatctccagagtggaacccgaggacctgggcgtgtactactgtctgcagagcacccactttccactgacctttggctccggcaccaagctggaaatcaagagagctgacgccgctcctaccgtgtccatctttccacctagcacagagcagctggccacaggcggagcatctgtcgtgtgcctgatgaacaacttctaccccagagacatcagcgtgaagtggaagatcgacggcaccgagagaagagatggcgtgctggatagcgtgaccgaccaggacagcaaggactccacctactccatgagcagcaccctgagcctgaccaaggccgattacgagagccacaacctgtacacatgcgaggtggtgcacaagaccagcagcagccctgtggtcaagagcttcaaccggaacgagtgctga

SEQ ID NO: 11 - DNA, 48 bp, synthetic construct
  source 1..48: mol_type = other DNA
agaagcagccagagcctggtgcacagcgacggcaatacctacctgcac

SEQ ID NO: 12 - DNA, 21 bp, synthetic construct
  source 1..21: mol_type = other DNA
agagtgtccaaccggttcagc

SEQ ID NO: 13 - DNA, 27 bp, synthetic construct
  source 1..27: mol_type = other DNA
ctgcagagcacccactttccactgacc

SEQ ID NO: 14 - DNA, 1383 bp, synthetic construct
  source 1..1383: mol_type = other DNA
atggaatttggcctgtcctgggtgttcctggtggccctgtttagaggcgtgcagtgcgaagtgcagctggaagaatctggcggaggactggtccagcctggcagatctatgaagctgtcttgtgccgcctccggcttcaccttctctgattatggaatggcctgggtgctgcagggccctaccaaaggattggagtgggtcgcctctatctcctacgacggcaaccggccttactaccgggattccgtgaagggcagattcaccatctctcgggacaacgccaagagcaccctgtacctgcagatggaatccctgagatctgaggacaccgccacctactactgcgtgaaggatctgttcgagatcggcgacttcgattactggggacagggcgtgatggtcaccgtgtcctctgctgagacaaccgctccttctgtgtatcccctggctcctggcaccgctctgaagtccaattctatggtcaccctgggctgcctggtcaagggctattttcctgagcctgtgaccgtgacctggaactctggtgctctgtctagcggagtgcacacctttccagctgtgctgcagtctggcctgtacaccctgacatcctccgtgaccgtgcctagctctacatggtctagccaggccgtgacatgcaacgtggcccatcctgcctcttccaccaaggtggacaagaaaatcgtgcccagagagtgcaacccttgcggctgtacaggatctgaggtgtcctccgtgttcatcttcccacctaagaccaaggacgtgctcaccatcacactgacccctaaagtgacctgcgtggtggtggacatctcccagaatgaccctgaagtgcggttctcctggttcatcgacgacgtggaagtgcacacagctcagacccatgctcctgagaagcagtccaactccacactgagatccgtgtccgagctgcccatcgtgcatagagattggctgaacggcaagaccttcaagtgcaaagtgaactccggcgcctttcctgctcctatcgagaagtccatctccaagcctgagggcacccctagaggaccccaggtttacaccatggctcctccaaaagaagagatgacccagagccaggtgtccatcacctgtatggttaagggcttctaccctcctgacatctacaccgagtggaaaatgaacggccagcctcaagagaactacaagaacacccctcctaccatggataccgacggctcctacttcctgtactccaagctgaacgtgaagaaagagacatggcagcagggcaacaccttcacctgttccgtgctgcacgagggcctgcacaatcaccataccgagaagtctctgtcccactctcctggcaagtga

SEQ ID NO: 15 - DNA, 21 bp, synthetic construct
  source 1..21: mol_type = other DNA
ggcttcaccttctctgattat

SEQ ID NO: 16 - DNA, 18 bp, synthetic construct
  source 1..18: mol_type = other DNA
tcctacgacggcaaccgg

SEQ ID NO: 17 - DNA, 30 bp, synthetic construct
  source 1..30: mol_type = other DNA
gatctgttcgagatcggcgacttcgattac

SEQ ID NO: 18 - protein, 12 aa, synthetic construct
AKGEVPKDRFSA

SEQ ID NO: 19 - protein, 12 aa, synthetic construct
DAGEVPKDRFSA

SEQ ID NO: 20 - protein, 12 aa, synthetic construct
DKAEVPKDRFSA

SEQ ID NO: 21 - protein, 12 aa, synthetic construct
DKGAVPKDRFSA

SEQ ID NO: 22 - protein, 12 aa, synthetic construct
DKGEAPKDRFSA

SEQ ID NO: 23 - protein, 12 aa, synthetic construct
DKGEVAKDRFSA

SEQ ID NO: 24 - protein, 12 aa, synthetic construct
DKGEVPADRFSA

SEQ ID NO: 25 - protein, 12 aa, synthetic construct
DKGEVPKARFSA

SEQ ID NO: 26 - protein, 12 aa, synthetic construct
DKGEVPKDAFSA

SEQ ID NO: 27 - protein, 12 aa, synthetic construct
DKGEVPKDRASA

SEQ ID NO: 28 - protein, 12 aa, synthetic construct
DKGEVPKDRFAA

SEQ ID NO: 29 - protein, 12 aa, synthetic construct
DKGEVPKDRFSG

SEQ ID NO: 30 - protein, 241 aa, synthetic construct
MDMRVPAQLLGLLLLWLSGARCDVLMTQTPVSLPVSLGGQVSISCRSSQSLVHSDGNTYLHWYLQKPGQSPQLLIYRVSNRFSGVPDRFTGSGSGTDFTLKISRVEPEDLGVYYCLQSTHFPLTFGSGTKLEIKRTVAAPSVFIFPPSDEQLKSGTASVVCLLNNFYPREAKVQWKVDNALQSGNSQESVTEQDSKDSTYSLSSTLTLSKADYEKHKVYACEVTHQGLSSPVTKSFNRGEC

SEQ ID NO: 31 - protein, 468 aa, synthetic construct
MEFGLSWVFLVALFRGVQCEVQLVESGGGLVQPGRSMKLSCAASGFTFSDYGMAWVLQGPTKGLEWVASISYDGNRPYYRDSVKGRFTISRDNAKSTLYLQMESLRSEDTATYYCVKDLFEIGDFDYWGQGVMVTVSSASTKGPSVFPLAPSSKSTSGGTAALGCLVKDYFPEPVTVSWNSGALTSGVHTFPAVLQSSGLYSLSSVVTVPSSSLGTQTYICNVNHKPSNTKVDKKVEPKSCDKTHTCPPCPAPELLGGPSVFLFPPKPKDTLMISRTPEVTCVVVDVSHEDPEVKFNWYVDGVEVHNAKTKPREEQYNSTYRVVSVLTVLHQDWLNGKEYKCKVSNKALPAPIEKTISKAKGQPREPQVYTLPPSREEMTKNQVSLTCLVKGFYPSDIAVEWESNGQPENNYKTTPPVLDSDGSFFLYSKLTVDKSRWQQGNVFSCSVMHEALHNHYTQKSLSLSPGK

SEQ ID NO: 32 - DNA, 726 bp, synthetic construct
  source 1..726: mol_type = other DNA
atggacatgagagtgcctgctcagctgctgggactgctgctgctttggcttagcggcgccagatgtgacgtgctgatgacccagacacctgtgtctctgccagtgtctctcggaggccaggtgtccatcagctgtagaagcagccagagcctggtgcacagcgacggcaatacctacctgcactggtatctgcagaagcccggccagtctccacagctgctgatctacagagtgtccaaccggttcagcggcgtgcccgatagattcacaggatctggcagcggcaccgacttcaccctgaagatctccagagtggaacccgaggacctgggcgtgtactactgtctgcagagcacccactttccactgacctttggctccggcaccaagctggaaatcaagcggacagtggccgctcctagcgtgttcatctttccacctagcgacgagcagctgaagtctggcacagcctctgtcgtgtgcctgctgaacaacttctaccccagagaagccaaggtgcaatggaaggtggacaacgccctgcagagcggcaatagccaagagagcgtgaccgagcaggacagcaaggactctacctacagcctgagcagcaccctgacactgagcaaggccgactacgagaagcacaaagtgtacgcctgcgaagtgacccaccagggcctttctagccctgtgaccaagagcttcaaccggggcgagtgttga

SEQ ID NO: 33 - DNA, 1407 bp, synthetic construct
  source 1..1407: mol_type = other DNA
atggaatttggcctgagctgggtgttcctggtggccctgtttagaggcgtgcagtgcgaagtgcagctggtggaatctggcggaggactggttcagcctggcagatccatgaagctgagctgtgccgccagcggcttcacctttagcgattatggaatggcctgggtgctgcagggccctaccaaaggacttgagtgggtcgccagcatcagctacgacggcaacagaccctactaccgggacagcgtgaagggcagattcaccatcagccgggacaacgccaagagcaccctgtacctgcagatggaaagcctgagaagcgaggacaccgccacctactactgcgtgaaggacctgttcgagatcggcgacttcgactattggggccagggcgtgatggtcacagtgtctagcgccagcacaaagggccctagcgttttcccactggctcccagcagcaagtctacaagcggaggaacagccgctctgggctgcctggtcaaggattactttcccgagcctgtgaccgtgtcctggaatagcggagcactgacaagcggcgtgcacacctttccagctgtgctgcaaagcagcggcctgtactctctgagcagcgtcgtgacagtgcctagcagctctctgggcacccagacctacatctgcaatgtgaaccacaagcctagcaacaccaaggtggacaagaaggtggaacccaagagctgcgacaagacccacacctgtcctccatgtcctgctccagaactgctcggcggaccttccgtgttcctgtttcctccaaagcctaaggacaccctgatgatcagcagaacccctgaagtgacctgcgtggtggtggatgtgtctcacgaggaccccgaagtgaagttcaattggtacgtggacggcgtggaagtgcacaatgccaagaccaagcctagagaggaacagtacaacagcacctacagagtggtgtccgtgctgaccgtgctgcaccaggattggctgaacggcaaagagtacaagtgcaaggtgtccaacaaggccctgcctgctcctatcgagaaaaccatcagcaaggccaagggccagcctagggaaccccaggtttacacactgcctccaagccgggaagagatgaccaagaaccaggtgtccctgacctgcctcgtgaagggattctacccctccgatatcgccgtggaatgggagagcaatggccagccagagaacaactacaagacaacccctcctgtgctggacagcgacggctcattcttcctgtacagcaagctgacagtggacaagtccagatggcagcagggcaacgtgttcagctgcagcgtgatgcacgaggccctgcacaaccactacacccagaagtccctgagcctgtctcctggcaagtga

SEQ ID NO: 34 - protein, 241 aa, synthetic construct
MDMRVPAQLLGLLLLWLSGARCDVVMTQTPLSLPVTLGQPASISCRSSQSLVHSDGNTYLHWYLQKPGQSPQLLIYRVSNRFSGVPDRFSGSGSGTDFTLKISRVEAEDVGVYYCLQSTHFPLTFGQGTKLEIKRTVAAPSVFIFPPSDEQLKSGTASVVCLLNNFYPREAKVQWKVDNALQSGNSQESVTEQDSKDSTYSLSSTLTLSKADYEKHKVYACEVTHQGLSSPVTKSFNRGEC

SEQ ID NO: 35 - protein, 468 aa, synthetic construct
MEFGLSWVFLVALFRGVQCQVQLVESGGGVVQPGRSLRLSCAASGFTFSDYGMHWVRQAPGKGLEWVAVISYDGNRKYYADSVKGRFTISRDNSKNTLYLQMNSLRAEDTAVYYCAKDLFEIGDFDYWGQGTLVTVSSASTKGPSVFPLAPSSKSTSGGTAALGCLVKDYFPEPVTVSWNSGALTSGVHTFPAVLQSSGLYSLSSVVTVPSSSLGTQTYICNVNHKPSNTKVDKKVEPKSCDKTHTCPPCPAPELLGGPSVFLFPPKPKDTLMISRTPEVTCVVVDVSHEDPEVKFNWYVDGVEVHNAKTKPREEQYNSTYRVVSVLTVLHQDWLNGKEYKCKVSNKALPAPIEKTISKAKGQPREPQVYTLPPSREEMTKNQVSLTCLVKGFYPSDIAVEWESNGQPENNYKTTPPVLDSDGSFFLYSKLTVDKSRWQQGNVFSCSVMHEALHNHYTQKSLSLSPGK

SEQ ID NO: 36 - DNA, 726 bp, synthetic construct
  source 1..726: mol_type = other DNA
atggacatgagagtgcctgctcagctgctgggactgctgctgctttggcttagcggcgccagatgtgacgtggtcatgacacagacccctctgagcctgcctgtgacactgggacagcctgccagcatcagctgtagaagcagccagagcctggtgcacagcgacggcaatacctacctgcactggtatctgcagaagcccggccagtctccacagctgctgatctacagagtgtccaaccggttcagcggcgtgcccgatagattttctggcagcggctctggcaccgacttcaccctgaagatctccagagtggaagccgaggacgtgggcgtgtactactgtctgcagagcacccactttccactgacctttggccagggcaccaagctggaaatcaagcggacagtggccgctcctagcgtgttcatctttccacctagcgacgagcagctgaagtccggcacagcctctgttgtgtgcctgctgaacaacttctaccccagagaagccaaggtgcaatggaaggtggacaacgccctgcagagcggcaatagccaagagagcgtgaccgagcaggacagcaaggactctacctacagcctgagcagcaccctgacactgagcaaggccgactacgagaagcacaaagtgtacgcctgcgaagtgacccaccagggcctttctagccctgtgaccaagagcttcaaccggggcgagtgttga

SEQ ID NO: 37 - DNA, 1407 bp, synthetic construct
  source 1..1407: mol_type = other DNA
atggaatttggcctgagctgggtgttcctggtggccctgtttagaggcgtgcagtgtcaggtgcagctggtggaatctggtggcggagttgtgcagcctggcagaagcctgagactgtcttgtgccgccagcggcttcaccttcagcgattatggcatgcactgggtccgacaggcccctggcaaaggacttgaatgggtcgccgtgatcagctacgacggcaacagaaagtactacgccgacagcgtgaagggcagattcaccatcagccgggacaacagcaagaacaccctgtacctgcagatgaacagcctgagagccgaggacaccgccgtgtactactgtgccaaggacctgttcgagatcggcgacttcgattactggggccagggcacactggtcacagtgtctagcgccagcacaaagggccctagcgttttcccactggctcccagcagcaagtctacaagcggaggaacagccgctctgggctgcctggtcaaggattactttcccgagcctgtgaccgtgtcctggaatagcggagcactgacaagcggcgtgcacacctttccagctgtgctgcaaagcagcggcctgtactctctgagcagcgtcgtgacagtgcctagcagctctctgggcacccagacctacatctgcaatgtgaaccacaagcctagcaacaccaaggtggacaagaaggtggaacccaagagctgcgacaagacccacacctgtcctccatgtcctgctccagaactgctcggcggaccttccgtgttcctgtttcctccaaagcctaaggacaccctgatgatcagcagaacccctgaagtgacctgcgtggtggtggatgtgtctcacgaggaccccgaagtgaagttcaattggtacgtggacggcgtggaagtgcacaacgccaagaccaagcctagagaggaacagtacaacagcacctacagagtggtgtccgtgctgaccgtgctgcaccaggattggctgaacggcaaagagtacaagtgcaaggtgtccaacaaggccctgcctgctcctatcgagaaaaccatcagcaaggccaagggccagcctagggaaccccaggtttacacactgcctccaagccgggaagagatgaccaagaaccaggtgtccctgacctgcctcgtgaagggattctacccctccgatatcgccgtggaatgggagagcaatggccagccagagaacaactacaagacaacccctcctgtgctggacagcgacggctcattcttcctgtacagcaagctgacagtggacaagtccagatggcagcagggcaacgtgttcagctgcagcgtgatgcacgaggccctgcacaaccactacacccagaagtccctgagcctgtctcctggcaagtga

SEQ ID NO: 38 - protein, 129 aa, synthetic construct
MKSLRVLLVILWLQLSWVWSQQKEVEQNSGPLSVPEGAIASLNCTYSDRGSQSFFWYRQYSGKSPELIMFIYSNGDKEDGRFTAQLNKASQYVSLLIRDSQPSDSATYLCAADDKIIFGKGTRLHILPN

SEQ ID NO: 39 - protein, 140 aa, synthetic construct
IQNPDPAVYQLRDSKSSDKSVCLFTDFDSQTNVSQSKDSDVYITDKTVLDMRSMDFKSNSAVAWSNKSDFACANAFNNSIIPEDTFFPSSDVPCDVKLVEKSFETDTNLNFQNLSVIGFRILLLKVAGFNLLMTLRLWSS

SEQ ID NO: 40 - protein, 131 aa, synthetic construct
MGSWTLCCVSLCILVAKHTDAGVIQSPRHEVTEMGQEVTLRCKPISGHDYLFWYRQTMMRGLELLIYFNNNVPIDDSGMPEDRFSAKMPNASFSTLKIQPSEPRDSAVYFCASSRGGSGYTFGSGTRLTVV

SEQ ID NO: 41 - protein, 195 aa, synthetic construct
EDLNKVFPPEVAVFEPSKAEIAHTQKATLVCLATGFFPDHVELSWWVNGKEVHSGVSTDPQPLKEQPAGSGDKGEVPKDRFSAGSGLNDSRYCLSSRLRVSATFWQNPRNHFRCQVQFYGLSENDEWTQDRAKPVTQIVSAEAWGRADCGITSASYHQGVLSATILYEILLGKATLYAVLVSALVLMAMVKRKDF

SEQ ID NO: 42 - protein, 134 aa, synthetic construct
MEKMLECAFIVLWLQLGWLSGEDQVTQSPEALRLQEGESSSLNCSYTVSGLRGLFWYRQDPGKGPEFLFTLYSAGEEKEKERLKATLTKKESFLHITAPKPEDSATYLCAVHSTAQAGTALIFGKGTTLSVSSN

SEQ ID NO: 43 - protein, 140 aa, synthetic construct
IQNPDPAVYQLRDSKSSDKSVCLFTDFDSQTNVSQSKDSDVYITDKCVLDMRSMDFKSNSAVAWSNKSDFACANAFNNSIIPEDTFFPSSDVPCDVKLVEKSFETDTNLNFQNLSVIGFRILLLKVAGFNLLMTLRLWSS

SEQ ID NO: 44 - protein, 134 aa, synthetic construct
MGFRLLCCVAFCLLGAGPVDSGVTQTPKHLITATGQRVTLRCSPRSGDLSVYWYQQSLDQGLQFLIQYYNGEERAKGNILERFSAQQFPDLHSELNLSSLELGDSALYFCASSTHRGQTNYGYTFGSGTRLTVV

SEQ ID NO: 45 - protein, 195 aa, synthetic construct
EDLNKVFPPEVAVFEPSKAEIAHTQKATLVCLATGFFPDHVELSWWVNGKEVHSGVCTDPQPLKEQPAGSGDKGEVPKDRFSAGSGLNDSRYCLSSRLRVSATFWQNPRNHFRCQVQFYGLSENDEWTQDRAKPVTQIVSAEAWGRADCGITSASYHQGVLSATILYEILLGKATLYAVLVSALVLMAMVKRKDF

SEQ ID NO: 46 - protein, 134 aa, synthetic construct
MASAPISMLAMLFTLSGLRAQSVAQPEDQVNVAEGNPLTVKCTYSVSGNPYLFWYVQYPNRGLQFLLKYITGDNLVKGSYGFEAEFNKSQTSFHLKKPSALVSDSALYFCAVTREAQGGKLIFGQGTELSVKPN

SEQ ID NO: 47 - protein, 140 aa, synthetic construct; identical to SEQ ID NO: 39

SEQ ID NO: 48 - protein, 133 aa, synthetic construct
MGPGLLCWVLLCLLGAGPVDAGVTQSPTHLIKTRGQHVTLRCSPISGHKSVSWYQQVLGQGPQFIFQYYEKEERGRGNFPDRFSARQFPNYSSELNVNALLLGDSALYLCASSLSGDFNQPQHFGDGTRLSIL

SEQ ID NO: 49 - protein, 195 aa, synthetic construct; identical to SEQ ID NO: 41

SEQ ID NO: 50 - DNA, 387 bp, synthetic construct
  source 1..387: mol_type = other DNA
atgaagtccctgagagtgctgctggtcatcctgtggctgcagctgtcttgggtctggtcccagcagaaagaggtggaacagaacagcggccctctgtctgttcctgaaggcgctatcgcctctctgaattgcacctacagcgacagaggcagccagagcttcttctggtatcggcagtacagcggcaagagccccgagctgatcatgttcatctacagcaacggcgacaaagaggacggccggtttacagcccagctgaacaaagccagccagtacgtgtccctgctgatcagagattcccagccaagcgactccgccacctacctgtgtgccgccgacgacaagatcatcttcggcaagggaaccagactgcacatcctgcctaac

SEQ ID NO: 51 - DNA, 423 bp, synthetic construct
  source 1..423: mol_type = other DNA
attcagaaccccgatcctgccgtgtaccagctgagagacagcaagagcagcgacaagagcgtgtgtctgttcaccgacttcgacagccagaccaacgtgtcccagagcaaggacagcgacgtgtacatcaccgacaagaccgtgctggacatgcggagcatggacttcaagagcaacagcgccgtggcctggtccaacaagagcgatttcgcctgcgccaacgccttcaacaatagcattatccccgaggacacattcttccccagctccgatgtgccctgcgacgtgaagctggtggaaaagagcttcgagacagacaccaacctgaacttccagaacctgagcgtgatcggcttcagaatcctgctgctgaaggtggccggcttcaatctgctgatgaccctgagactgtggtccagctga

SEQ ID NO: 52 - DNA, 393 bp, synthetic construct
  source 1..393: mol_type = other DNA
atgggaagctggaccctgtgttgtgtgtccctgtgtatcctggtggccaagcacacagatgccggcgtgatccagtctcctagacacgaagtgaccgagatgggccaagaagtgaccctgcgctgcaagcctatcagcggccacgattacctgttctggtacagacagaccatgatgagaggcctggaactgctgatctacttcaacaacaacgtgcccatcgacgacagcggaatgcccgaggatagattcagcgccaagatgcccaacgccagcttcagcaccctgaagatccagcctagcgagcccagagatagcgccgtgtacttttgcgcctcttccagaggcggcagcggctacacatttggctctggcacaagactgaccgtggtg

SEQ ID NO: 53 - DNA, 585 bp, synthetic construct
  source 1..585: mol_type = other DNA
gaagatctgaacaaggtgttccctccagaggtggccgtgttcgagccttctaaggccgagattgcccacacacagaaagccacactcgtgtgcctggctaccggcttctttcctgaccacgtggaactgtcttggtgggtcaacggcaaagaggtgcacagcggcgtcagcacagatccccagcctctgaaagaacagcccgctggatctggcgataagggcgaagtgcccaaggacagattttccgccggatctggactgaacgacagccggtactgtctgagcagcagactgagagtgtccgccacattctggcagaaccccagaaaccacttcagatgccaggtgcagttctacggcctgagcgagaacgatgagtggacccaggatagagccaagcctgtgacacagatcgtgtctgccgaagcctggggcagagccgattgtggaattaccagcgccagctaccatcagggcgtgctgtctgccacaatcctgtacgagatcctgctgggcaaagccactctgtacgccgtgctggtgtctgccctggtgctgatggccatggtcaagagaaaggacttt

SEQ ID NO: 54 - DNA, 402 bp, synthetic construct
  source 1..402: mol_type = other DNA
atggaaaagatgctggaatgcgccttcatcgtgctgtggctgcagctgggatggctgagcggagaggaccaagtgacccagtctcccgaggccctgagactgcaggaaggcgagagcagcagcctgaattgcagctacaccgtgtccggcctgcggggcctgttctggtatagacaggaccctggcaagggccccgagttcctgtttaccctgtactctgccggcgaagagaaagaaaaagagcggctgaaggccacactgaccaagaaagagagcttcctgcacatcaccgcccccaagcctgaggacagcgccacatatctgtgcgccgtgcactctacagcccaggccggaaccgccctgatcttcggcaagggcacaaccctgtccgtgtccagcaac

SEQ ID NO: 55 - DNA, 423 bp, synthetic construct
  source 1..423: mol_type = other DNA
atccagaaccccgaccccgccgtgtaccagctgagagacagcaagagcagcgacaagagcgtgtgcctgttcaccgacttcgacagccagacaaacgtgtcccagagcaaggacagcgacgtgtacatcaccgataagtgcgtgctggacatgcggagcatggacttcaagagcaacagcgccgtggcctggtccaacaagagcgatttcgcctgcgccaacgccttcaacaacagcattatccccgaggacacattcttccccagctccgacgtgccctgcgacgtgaagctggtggaaaagagcttcgagacagacaccaacctgaacttccagaatctgagcgtgatcggcttcagaatcctgctgctgaaggtggccggcttcaatctgctgatgaccctgcggctgtggtccagctga

SEQ ID NO: 56 - DNA, 402 bp, synthetic construct
  source 1..402: mol_type = other DNA
atgggcttccggctgctgtgttgcgtggccttctgtctgctgggagccggccctgtggatagcggcgtgacacagacacccaagcacctgatcaccgccaccggccagcgcgtgacactgagatgtagccctagaagcggcgacctgagcgtgtactggtatcagcagagcctggaccagggcctgcagttcctgatccagtactacaacggcgaggaacgggccaagggcaacatcctggaacggttcagcgcccagcagttccccgatctgcacagcgagctgaacctgagcagcctggaactgggcgacagcgccctgtacttctgtgccagcagcacccacagaggccagaccaactacggctacaccttcggcagcggcaccagactgaccgtggtg

SEQ ID NO: 57 - DNA, 585 bp, synthetic construct
  source 1..585: mol_type = other DNA
gaagatctgaacaaggtgttccccccagaggtggccgtgttcgagcctagcaaggccgagatcgcccacacccagaaagccaccctcgtgtgtctggccaccggctttttccccgaccacgtggaactgtcttggtgggtcaacggcaaagaggtgcactccggcgtgtgcaccgatccccagcctctgaaagaacagcccgccggatctggcgataagggcgaagtgcccaaggacagattttccgccggatctggactgaacgacagccggtactgcctgtccagcagactgagagtgtccgccaccttctggcagaacccccggaaccacttcagatgccaggtgcagttctacggcctgagcgagaacgacgagtggacccaggacagagccaagcccgtgacccagatcgtgtctgccgaagcctggggcagagccgattgtggcatcaccagcgccagctaccatcagggcgtgctgagcgccaccatcctgtacgagatcctgctgggcaaggccaccctgtacgccgtgctggtgtctgccctggtgctgatggccatggtcaagcggaaggacttt

SEQ ID NO: 58 - DNA, 402 bp, synthetic construct
  source 1..402: mol_type = other DNA
atggccagcgctcctattagcatgctggccatgctgttcaccctgtccggactgagagcacagtctgtggcccagcctgaggaccaagtgaatgtggccgagggcaatcccctgaccgtgaagtgtacctacagcgtgtccggcaatccctacctgttttggtacgtgcagtaccccaaccggggcctgcagttcctgctgaagtacatcaccggcgacaacctggtcaagggcagctatggattcgaggccgagttcaacaagagccagaccagcttccacctgaagaaacccagcgctctggtgtctgactctgccctgtacttctgcgccgtgaccagagaagcccaaggcggcaagctgatctttggccagggaacagagctgtccgtgaagcccaac

SEQ ID NO: 59 - DNA, 423 bp, synthetic construct
  source 1..423: mol_type = other DNA
attcagaaccccgatcctgccgtgtaccagctgagagacagcaagagcagcgacaagtccgtgtgtctgttcaccgacttcgactcccagaccaacgtgtcccagagcaaggacagcgacgtgtacatcacagacaagaccgtgctggacatgcggagcatggacttcaagagcaacagcgccgtggcctggtccaacaagtccgatttcgcctgcgccaacgccttcaacaacagcattatccccgaggacacattcttccccagctccgatgtgccctgcgacgtgaagctggtggaaaagagcttcgagacagacaccaacctgaacttccagaacctgagcgtgatcggcttcagaatcctgctgctgaaggtggccggcttcaatctgctgatgaccctgcgactgtggtccagctaa

SEQ ID NO: 60 - DNA, 399 bp, synthetic construct
  source 1..399: mol_type = other DNA
atgggacccggcctgctgtgttgggttctgctgtgtctgcttggagccggacctgtggatgctggcgttacacagtctcccacacacctgatcaagaccagaggccagcacgtgaccctgagatgctctcctatcagcggccacaagagcgtgtcctggtatcagcaggttctcggccagggacctcagttcatcttccagtactacgagaaagaggaacgcggcagaggcaacttccccgacagattttccgccagacagttccccaactacagctccgagctgaacgtgaacgctctgctgctgggagatagcgccctgtacctgtgtgcctctagcctgagcggcgacttcaatcagcctcagcactttggcgacggcaccagactgagcatcctg

SEQ ID NO: 61 - DNA, 585 bp, synthetic construct
  source 1..585: mol_type = other DNA
gaagatctgaacaaggtgttccctccagaggtggccgtgttcgagccttctaaggccgagattgcccacacacagaaagccacactcgtgtgcctggccaccggctttttccccgatcacgtcgaactgtcttggtgggtcaacggcaaagaggtgcacagcggcgtcagcacagatccccagcctctgaaagaacagcctgccggctctggcgataagggcgaagtgcccaaggatagattcagcgccggcagcggcctgaacgacagcagatattgtctgagcagcagactgcgggtgtccgccaccttttggcagaaccccagaaaccacttcagatgccaggtgcagttctacggcctgagcgagaacgatgagtggacccaggatagagccaagcctgtgacacagatcgtgtctgccgaagcctggggcagagccgattgtggaattaccagcgccagctaccatcagggcgtgctgtctgccacaatcctgtacgagatcctgctgggcaaagccactctgtacgccgtgctggtttctgccctggtgctgatggccatggtcaagagaaaggacttt

SEQ ID NO: 62 - protein, 6 aa, synthetic construct
  VARIANT 5: note = X may be A, R, N, D, C, Q, E, G, H, I, L, K, M, F, P, S, T, W, Y, V
EVPKXR

SEQ ID NO: 63 - protein, 9 aa, synthetic construct
  VARIANT 6: note = X may be A, R, N, D, C, Q, E, G, H, I, L, K, M, F, P, S, T, TW, Y, V
GEVPKXRFS

SEQ ID NO: 64 - protein, 12 aa, synthetic construct
  VARIANT 1: note = X is selected from D and E
  VARIANT 2: note = X is selected from K, R, H
  VARIANT 8: note = X is selected from A, R, N, D, C, Q, E, G, H, I, L, K, M, F, P, S, T, W, Y, V
  VARIANT 12: note = X is selected from G, L, A, V, M, I, S, T
XXGEVPKXRFSX

SEQ ID NO: 65 - protein, 12 aa, synthetic construct
  VARIANT 2: note = X is selected from K, R, H
  VARIANT 8: note = X is selected from A, R, N, D, C, Q, E, G, H, I, L, K, M, F, P, S, T, W, Y, V
  VARIANT 12: note = X is selected from G, L, A, V, M, I, S, T
DXGEVPKXRFSX

SEQ ID NO: 66 - protein, 12 aa, synthetic construct
  VARIANT 2: note = X is seleceted from K, R, and H
  VARIANT 8: note = X is selected from A, R, N, D, C, Q, E, G, H, I, L, K, M, F, P, S, T, W, Y, V
  VARIANT 12: note = X is selected from G, L, A, V, M, I, S, and T
EXGEVPKXRFSX

SEQ ID NO: 67 - protein, 12 aa, synthetic construct
  VARIANT 1: note = X is selected from D and E
  VARIANT 8: note = X is selected from A, R, N, D, C, Q, E, G, H, I, L, K, M, F, P, S, T, W, Y, V
  VARIANT 12: note = X is selected from G, L, A, V, M, I, S, and T
XKGEVPKXRFSX

SEQ ID NO: 68 - protein, 12 aa, synthetic construct
  VARIANT 1: note = X is selected from D and E
  VARIANT 8: note = X is selected from A, R, N, D, C, Q, E, G, H, I, L, K, M, F, P, S, T, W, Y, V
  VARIANT 12: note = X is selected from G, L, A, V, M, I, S, and T
XRGEVPKXRFSX

SEQ ID NO: 69 - protein, 12 aa, synthetic construct
  VARIANT 1: note = X is selected from D and E
  VARIANT 8: note = X is selected from A, R, N, D, C, Q, E, G, H, I, L, K, M, F, P, S, T, W, Y, V
  VARIANT 12: note = X is selected from G, L, A, V, M, I, S, and T
XHGEVPKXRFSX

SEQ ID NO: 70 - protein, 12 aa, synthetic construct
  VARIANT 1: note = X is selected from D and E
  VARIANT 2: note = X is selected from K, R, and H
  VARIANT 8: note = X is selected from A, R, N, D, C, Q, E, G, H, I, L, K, M, F, P, S, T, W, Y, V
XXGEVPKXRFSG

SEQ ID NO: 71 - protein, 12 aa, synthetic construct
  VARIANT 1: note = X is selected from D and E
  VARIANT 2: note = X is selected from K, R, and H
  VARIANT 8: note = X is selected from A, R, N, D, C, Q, E, G, H, I, L, K, M, F, P, S, T, W, Y, V
XXGEVPKXRFSL

SEQ ID NO: 72 - protein, 12 aa, synthetic construct
  VARIANT 1: note = X is selected from D and E
  VARIANT 2: note = X is selected from K, R, and H
  VARIANT 8: note = X is selected from A, R, N, D, C, Q, E, G, H, I, L, K, M, F, P, S, T, W, Y, V
XXGEVPKXRFSA

SEQ ID NO: 73 - protein, 12 aa, synthetic construct
  VARIANT 1: note = X is selected from D and E
  VARIANT 2: note = X is selected from K, R, and H
  VARIANT 8: note = X is selected from A, R, N, D, C, Q, E, G, H, I, L, K, M, F, P, S, T, W, Y, V
XXGEVPKXRFSV

SEQ ID NO: 74 - protein, 12 aa, synthetic construct
  VARIANT 1: note = X is selected from D and E
  VARIANT 2: note = X is selected from K, R, and H
  VARIANT 8: note = X is selected from A, R, N, D, C, Q, E, G, H, I, L, K, M, F, P, S, T, W, Y, V
XXGEVPKXRFSM

SEQ ID NO: 75 - protein, 12 aa, synthetic construct
  VARIANT 1: note = X is selected from D and E
  VARIANT 2: note = X is selected from K, R, and H
  VARIANT 8: note = X is selected from A, R, N, D, C, Q, E, G, H, I, L, K, M, F, P, S, T, W, Y, V
XXGEVPKXRFSI

SEQ ID NO: 76 - protein, 12 aa, synthetic construct
  VARIANT 1: note = X is selected from D and E
  VARIANT 2: note = X is selected from K, R, and H
  VARIANT 8: note = X is is selected from A, R, N, D, C, Q, E, G, H, I, L, K, M, F, P, S, T, W, Y, V
XXGEVPKXRFSS

SEQ ID NO: 77 - protein, 12 aa, synthetic construct
  VARIANT 1: note = X is selected from D and E
  VARIANT 2: note = X is selected from K, R, and H
  VARIANT 8: note = X is selected from A, R, N, D, C, Q, E, G, H, I, L, K, M, F, P, S, T, W, Y, V
XXGEVPKXRFST

SEQ ID NO: 78 - protein, 12 aa, synthetic construct
  VARIANT 8: note = X is selected from A, R, N, D, C, Q, E, G, H, I, L, K, M, F, P, S, T, W, Y, V
  VARIANT 12: note = X is selected from G, L, A, V, M, I, S, and T
DKGEVPKXRFSX

SEQ ID NO: 79 - protein, 12 aa, synthetic construct
  VARIANT 8: note = X is selected from A, R, N, D, C, Q, E, G, H, I, L, K, M, F, P, S, T, W, Y, V
  VARIANT 12: note = X is selected from G, L, A, V, M, I, S, and T
DRGEVPKXRFSX

SEQ ID NO: 80 - protein, 12 aa, synthetic construct
  VARIANT 8: note = X is selected from A, R, N, D, C, Q, E, G, H, I, L, K, M, F, P, S, T, W, Y, V
  VARIANT 12: note = X is selected from G, L, A, V, M, I, S, and T
DHGEVPKXRFSX

SEQ ID NO: 81 - protein, 12 aa, synthetic construct
  VARIANT 8: note = X is selected from A, R, N, D, C, Q, E, G, H, I, L, K, M, F, P, S, T, W, Y, V
  VARIANT 12: note = X is selected from G, L, A, V, M, I, S, and T
EKGEVPKXRFSX

SEQ ID NO: 82 - protein, 12 aa, synthetic construct
  VARIANT 8: note = X is selected from A, R, N, D, C, Q, E, G, H, I, L, K, M, F, P, S, T, W, Y, V
  VARIANT 12: note = X is selected from G, L, A, V, M, I, S, and T
ERGEVPKXRFSX

SEQ ID NO: 83 - protein, 12 aa, synthetic construct
  VARIANT 8: note = X is selected from A, R, N, D, C, Q, E, G, H, I, L, K, M, F, P, S, T, W, Y, V
  VARIANT 12: note = X is selected from G, L, A, V, M, I, S, and T
EHGEVPKXRFSX

SEQ ID NO: 84 - protein, 12 aa, synthetic construct
  VARIANT 8: note = X is selected from A, R, N, D, C, Q, E, G, H, I, L, K, M, F, P, S, T, W, Y, V
DKGEVPKXRFSA

SEQ ID NO: 85 - protein, 11 aa, synthetic construct
  VARIANT 7: note = X is selected from A, R, N, D, C, Q, E, G, H, I, L, K, M, F, P, S, T, W, Y, V
KGEVPKXRFSA

SEQ ID NO: 86 - protein, 10 aa, synthetic construct
  VARIANT 6: note = X is selected from A, R, N, D, C, Q, E, G, H, I, L, K, M, F, P, S, T, W, Y, V
GEVPKXRFSA

SEQ ID NO: 87 - protein, 9 aa, synthetic construct
  VARIANT 6: note = X is selected from A, R, N, D, C, Q, E, G, H, I, L, K, M, F, P, S, T, W, Y, V
GEVPKXRFS

SEQ ID NO: 88 - protein, 11 aa, synthetic construct
  VARIANT 8: note = X is selected from A, R, N, D, C, Q, E, G, H, I, L, K, M, F, P, S, T, W, Y, V
DKGEVPKXRFS

SEQ ID NO: 89 - protein, 9 aa, synthetic construct
  VARIANT 7: note = X is selected from A, R, N, D, C, Q, E, G, H, I, L, K, M, F, P, S, T, W, Y, V
KGEVPKXRF

SEQ ID NO: 90 - protein, 5 aa, synthetic construct
GGGGS